European Patent Application EP 4 198 046 A1, published June 21, 2023. Title: ALPHA-SARCOGLYCAN GENE TRANSFER INCREASE USING MODIFIED ITR SEQUENCES. Applicant: GENETHON INSTITUT NATIONAL DE LA SANTE ET DE LA RECHERCHE MEDICALE UNIVERSITE D'EVRY VAL D’ESSONNE. The sequence listing filed with the application follows.

SEQUENCE LISTING (11 sequences)

SEQ ID NO: 1 - DNA, 130 bp, Artificial Sequence
  ITRg 5'
ctgcgcgctcgctcgctcactgaggccgcccgggcaaagcccgggcgtcgggcgacctttggtcgcccggcctcagtgagcgagcgagcgcgcagagagggagtggccaactccatcactaggggttcct

SEQ ID NO: 2 - DNA, 130 bp, Artificial Sequence
  ITRg 3'
aggaacccctagtgatggagttggccactccctctctgcgcgctcgctcgctcactgaggccgggcgaccaaaggtcgcccgacgcccgggctttgcccgggcggcctcagtgagcgagcgagcgcgcag

SEQ ID NO: 3 - DNA, 1164 bp, Artificial Sequence
  SGCA WT
atggctgagacactcttctggactcctctcctcgtggttctcctggcagggctgggggacaccgaggcccagcagaccacgctacacccacttgtgggccgtgtctttgtgcacaccttggaccatgagacgtttctgagccttcctgagcatgtcgctgtcccacccgctgtccacatcacctaccacgcccacctccagggacacccagacctgccccggtggctccgctacacccagcgcagcccccaccaccctggcttcctctacggctctgccaccccagaagatcgtgggctccaggtcattgaggtcacagcctacaatcgggacagctttgataccactcggcagaggctggtgctggagattggggacccagaaggccccctgctgccataccaagccgagttcctggtgcgcagccacgatgcggaggaggtgctgccctcaacacctgccagccgcttcctctcagccttggggggactctgggagcccggagagcttcagctgctcaacgtcacctctgccttggaccgtgggggccgtgtcccccttcccattgagggccgaaaagaaggggtatacattaaggtgggttctgcctcacctttttctacttgcctgaagatggtggcatcccccgatagccacgcccgctgtgcccagggccagcctccacttctgtcttgctacgacaccttggcaccccacttccgcgttgactggtgcaatgtgaccctggtggataagtcagtgccggagcctgcagatgaggtgcccaccccaggtgatgggatcctggagcatgacccgttcttctgcccacccactgaggccccagaccgtgacttcttggtggatgctctggtcaccctcctggtgcccctgctggtggccctgcttctcaccttgctgctggcctatgtcatgtgctgccggcgggagggaaggctgaagagagacctggctacctccgacatccagatggtccaccactgcaccatccacgggaacacagaggagctgcggcagatggcggccagccgcgaggtgccccggccactctccaccctgcccatgttcaatgtgcacacaggtgagcggctgcctccccgcgtggacagcgcccaggtgcccctcattctggaccagcactga

SEQ ID NO: 4 - DNA, 1061 bp, Artificial Sequence
  Human Desmin Promoter
taccccctgccccccacagctcctctcctgtgccttgtttcccagccatgcgttctcctctataaatacccgctctggtatttggggttggcagctgttgctgccagggagatggttgggttgacatgcggctcctgacaaaacacaaacccctggtgtgtgtgggcgtgggtggtgtgagtagggggatgaatcagggagggggcgggggacccagggggcaggagccacacaaagtctgtgcgggggtgggagcgcacatagcaattggaaactgaaagcttatcagaccctttctggaaatcagcccactgtttataaacttgaggccccaccctcgacagtaccggggaggaagagggcctgcactagtccagagggaaactgaggctcagggctagctcgcccatagacatacatggcaggcaggctttggccaggatccctccgcctgccaggcgtctccctgccctcccttcctgcctagagacccccaccctcaagcctggctggtctttgcctgagacccaaacctcttcgacttcaagagaatatttaggaacaaggtggtttagggcctttcctgggaacaggccttgaccctttaagaaatgacccaaagtctctccttgaccaaaaaggggaccctcaaactaaagggaagcctctcttctgctgtctcccctgaccccactcccccccaccccaggacgaggagataaccagggctgaaagaggcccgcctgggggctgcagacatgcttgctgcctgccctggcgaaggattggcaggcttgcccgtcacaggacccccgctggctgactcaggggcgcaggcctcttgcgggggagctggcctccccgcccccacggccacgggccgccctttcctggcaggacagcgggatcttgcagctgtcaggggaggggaggcgggggctgatgtcaggagggatacaaatagtgccgacggctgggggccctgtctcccctcgccgcatccactctccggccggccgcctgcccgccgcctcctccgtgcgcccgccagcctcgcccgc

SEQ ID NO: 5 - DNA, 762 bp, Artificial Sequence
  pA-HBB2
accccaccagtgcaggctgcctatcagaaagtggtggctggtgtggctaatgccctggcccacaagtatcactaagctcgctttcttgctgtccaatttctattaaaggttcctttgttccctaagtccaactactaaactgggggatattatgaagggccttgagcatctggattctgcctaataaaaaacatttattttcattgcaatgatgtatttaaattatttctgaatattttactaaaaagggaatgtgggaggtcagtgcatttaaaacataaagaaatgaagagctagttcaaaccttgggaaaatacactatatcttaaactccatgaaagaaggtgaggctgcaaacagctaatgcacattggcaacagccctgatgcctatgccttattcatccctcagaaaaggattcaagtagaggcttgatttggaggttaaagttttgctatgctgtattttacattacttattgttttagctgtcctcatgaatgtcttttcactacccatttgcttatcctgcatctctcagccttgactccactcagttctcttgcttagagataccacctttcccctgaagtgttccttccatgttttacggcgagatggtttctcctcgcctggccactcagccttagttgtctctgttgtcttatagaggtctacttgaagaaggaaaaacagggggcatggtttgactgtcctgtgagcccttcttccctgcctcccccactcacagtgacccggaatc

SEQ ID NO: 6 - DNA, 18 bp, Artificial Sequence
  polyA HBB2 sequence FWD
ccaggcgaggagaaacca

SEQ ID NO: 7 - DNA, 25 bp, Artificial Sequence
  polyA HBB2 sequence REV
cttgactccactcagttctcttgct

SEQ ID NO: 8 - DNA, 29 bp, Artificial Sequence
  polyA HBB2 sequence Probe
ctcgccgtaaaacatggaaggaacacttc

SEQ ID NO: 9 - DNA, 20 bp, Artificial Sequence
  ribosomal phosphoprotein FWD
ctccaagcagatgcagcaga

SEQ ID NO: 10 - DNA, 20 bp, Artificial Sequence
  ribosomal phosphoprotein REV
atagccttgcgcatcatggt

SEQ ID NO: 11 - DNA, 22 bp, Artificial Sequence
  ribosomal phosphoprotein Probe
ccgtggtgctgatgggcaagaa